European Patent Application EP 4 729 537 A1, published April 22, 2026. Title: B-LACTAMASE-INHIBITING ANTIBODY AND USE THEREOF IN THE TREATMENT AND/OR PREVENTION OF INFECTIONS CAUSED BY B-LACTAMASE-PRODUCING BACTERIA. Applicant: Consejo Superior de Investigaciones Cientificas (CSIC). Application ES. The sequence listing filed with the application follows.

SEQUENCE LISTING (47 sequences)

SEQ ID NO: 1 - protein, 8 aa, synthetic construct
  source 1..8: note = CDR1 antibody B2; note (original language) = CDR1 anticuerpo B2; organism (original language) = construccion sintetica
GTIFVYPY

SEQ ID NO: 2 - protein, 14 aa, synthetic construct
  source 1..14: note = CDR2 antibody B2; note (original language) = CDR2 anticuerpo B2; organism (original language) = construccion sintetica
EFVAGIGQGATTYY

SEQ ID NO: 3 - protein, 18 aa, synthetic construct
  source 1..18: note = CDR3 antibody B2; note (original language) = CDR3 anticuerpo B2; organism (original language) = construccion sintetica
AYRYRDDVRRYGIDRYHT

SEQ ID NO: 4 - protein, 8 aa, synthetic construct
  source 1..8: note = CDR1 antibody B3; note (original language) = CDR1 anticuerpo B3; organism (original language) = construccion sintetica
GTIFYYPY

SEQ ID NO: 5 - protein, 14 aa, synthetic construct
  source 1..14: note = CDR2 antibody B3; note (original language) = CDR2 anticuerpo B3; organism (original language) = construccion sintetica
EFVAGIDYGSTTYY

SEQ ID NO: 6 - protein, 18 aa, synthetic construct
  source 1..18: note = CDR3 antibody B3; note (original language) = CDR3 anticuerpo B3; organism (original language) = construccion sintetica
VVYLVTRKGASQQDEIYS

SEQ ID NO: 7 - protein, 8 aa, synthetic construct
  source 1..8: note = CDR1 antibody B4; note (original language) = CDR1 anticuerpo B4; organism (original language) = contruccion sintetica
GTIFAQDY

SEQ ID NO: 8 - protein, 14 aa, synthetic construct
  source 1..14: note = CDR2 antibody B4; note (original language) = CDR2 anticuerpo B4; organism (original language) = construccion sintetica
EFVASIAYGTITYY

SEQ ID NO: 9 - protein, 10 aa, synthetic construct
  source 1..10: note = CDR3 antibody B4; note (original language) = CDR3 anticuerpo B4; organism (original language) = construccion sintetica
VYPTPVTDYI

SEQ ID NO: 10 - protein, 8 aa, synthetic construct
  source 1..8: note = CDR1 antibody B5; note (original language) = CDR1 anticuerpo B5; organism (original language) = construccion sintetica
GNISDLGT

SEQ ID NO: 11 - protein, 14 aa, synthetic construct
  source 1..14: note = CDR2 antibody B5; note (original language) = CDR2 anticuerpo B5; organism (original language) = construccion sintetica
EFVAGIGTGSNTYY

SEQ ID NO: 12 - protein, 12 aa, synthetic construct
  source 1..12: note = CDR3 antibody B5; note (original language) = CDR3 anticuerpo B5; organism (original language) = construccion sintetica
VIAGRSYWIYFY

SEQ ID NO: 13 - protein, 8 aa, synthetic construct
  source 1..8: note = CDR1 antibody B6; note (original language) = CDR1 anticuerpo B6; organism (original language) = construccion sintetica
GTISAVSG

SEQ ID NO: 14 - protein, 14 aa, synthetic construct
  source 1..14: note = CDR2 antibody B6; note (original language) = CDR2 anticuerpo B6; organism (original language) = construccion sintetica
EFVASINRGSTTNY

SEQ ID NO: 15 - protein, 10 aa, synthetic construct
  source 1..10: note = CDR3 antibody B6; note (original language) = CDR3 anticuerpo B6
ALHGTGRVHV

SEQ ID NO: 16 - protein, 127 aa, synthetic construct
  source 1..127: note = Antibody B2; note (original language) = Anticuerpo B2; organism (original language) = construccion sintetica
MQVQLQESGGGLVQAGGSLRLSCAASGTIFVYPYMGWYRQAPGKEREFVAGIGQGATTYYADSVKGRFTISRDNAKNTVYLQMNSLKPEDTAVYYCAAYRYRDDVRRYGIDRYHTYWGQGTQVTVSS

SEQ ID NO: 17 - protein, 127 aa, synthetic construct
  source 1..127: note = Antibody B3; note (original language) = Anticuerpo B3; organism (original language) = construccion sintetica
MQVQLQESGGGLVQAGGSLRLSCAASGTIFYYPYMGWYRQAPGKEREFVAGIDYGSTTYYADSVKGRFTISRDNAKNTVYLQMNSLKPEDTAVYYCAVVYLVTRKGASQQDEIYSYWGQGTQVTVSS

SEQ ID NO: 18 - protein, 119 aa, synthetic construct
  source 1..119: note = Antibody B4; note (original language) = Anticuerpo B4; organism (original language) = construccion sintetica
MQVQLQESGGGLVQAGGSLRLSCAASGTIFAQDYMGWYRQAPGKEREFVASIAYGTITYYADSVKGRFTISRDNAKNTVYLQMNSLKPEDTAVYYCAVYPTPVTDYIYWGQGTQVTVSS

SEQ ID NO: 19 - protein, 121 aa, synthetic construct
  source 1..121: note = Antibody B5; note (original language) = Anticuerpo B5; organism (original language) = construccion sintetica
MQVQLQESGGGLVQAGGSLRLSCAASGNISDLGTMGWYRQAPGKEREFVAGIGTGSNTYYADSVKGRFTISRDNAKNTVYLQMNSLKPEDTAVYYCAVIAGRSYWIYFYYWGQGTQVTVSS

SEQ ID NO: 20 - protein, 119 aa, synthetic construct
  source 1..119: note = Antibody B6; note (original language) = Anticuerpo B6; organism (original language) = construccion sintetica
MQVQLQESGGGLVQAGGSLRLSCAASGTISAVSGMGWYRQAPGKEREFVASINRGSTTNYADSVKGRFTISRDNAKNTVYLQMNSLKPEDTAVYYCAALHGTGRVHVYWGQGTQVTVSS

SEQ ID NO: 21 - protein, 259 aa, synthetic construct
  source 1..259: note = fragment Class A B-lactamase Mycobacterium abscessus; note (original language) = Fragmento de B-lactamasa de clase A Mycobacterium abscessus; organism (original language) = construccion sintetica
APDELASLEKDFGGRIGVYALDTGSGDTVGHRADERFLMCSTVKTFIVSAILRRRLSEPGLLDQRIQYTQSDVLEWAPITSQHVSTGMTVSELCDATLRYSDNTGANLLITQLGGPKETEKFVRSLGDNVTRMDRTEVQLNIPDGDLDTSTPQQLVANLRRLVLDEGLDSRGRDLLTDWLKRNTTGDQSIRAAVPAGWTVADKTGGGFKGETNDIAVIWPPGRAPIVMAVLTVPEDPTSTKGKPTIAAATRIVLRAFGA

SEQ ID NO: 22 - protein, 8 aa, synthetic construct
  source 1..8: note = CDR1 antibody B1; note (original language) = CDR1 anticuerpo B1; organism (original language) = construccion sintetica
GNIFTVSS

SEQ ID NO: 23 - protein, 14 aa, synthetic construct
  source 1..14: note = CDR2 antibody B1; note (original language) = CDR2 anticuerpo B1; organism (original language) = construccion sintetica
EFVAAISDGATTNY

SEQ ID NO: 24 - protein, 10 aa, synthetic construct
  source 1..10: note = CDR3 antibody B1; note (original language) = CD3 anticuerpo B1; organism (original language) = construccion sintetica
AYASRVGLTV

SEQ ID NO: 25 - protein, 6 aa, synthetic construct
  source 1..6: note = histidine tag; note (original language) = cola de histidina; organism (original language) = construccion sintetica
HHHHHH

SEQ ID NO: 26 - protein, 8 aa, synthetic construct
  source 1..8: note = CDR1 antibody B7; note (original language) = CDR1 anticuerpo B7; organism (original language) = construccion sintetica
GTISKAPV

SEQ ID NO: 27 - protein, 14 aa, synthetic construct
  source 1..14: note = CDR2 antibody B7; note (original language) = CDR2 anticuerpo B7; organism (original language) = construccion sintetica
EFVASINRGSTTNY

SEQ ID NO: 28 - protein, 14 aa, synthetic construct
  source 1..14: note = CDR3 antibody B7; note (original language) = CDR3 anticuerpo B7; organism (original language) = construccion sintetica
AYVHIRRSGYIALT

SEQ ID NO: 29 - protein, 119 aa, synthetic construct
  source 1..119: note = Antibody B1; note (original language) = Anticuerpo B1; organism (original language) = construccion sintetica
MQVQLQESGGGLVQAGGSLRLSCAASGNIFTVSSMGWYRQAPGKEREFVAAISDGATTNYADSVKGRFTISRDNAKNTVYLQMNSLKPEDTAVYYCAAYASRVGLTVYWGQGTQVTVSS

SEQ ID NO: 30 - protein, 123 aa, synthetic construct
  source 1..123: note = antibody B7; note (original language) = Anticuerpo B7; organism (original language) = construccion sintetica
MQVQLQESGGGLVQAGGSLRLSCAASGTISKAPVMGWYRQAPGKEREFVAGIASGSNTNYADSVKGRFTISRDNAKNTVYLQMNSLKPEDTAVYYCAAYVHIRRSGYIALTYWGQGTQVTVSS

SEQ ID NO: 31 - protein, 289 aa, Mycobacterium abscessus
  source 1..289: note = Class A B-lacatamase; note (original language) = B-lactamasa de clase A
MISRRALLVGGVSAVGVVAAGCSRNGNRRPAPDELASLEKDFGGRIGVYALDTGSGDTVGHRADERFLMCSTVKTFIVSAILRRRLSEPGLLDQRIQYTQSDVLEWAPITSQHVSTGMTVSELCDATLRYSDNTGANLLITQLGGPKETEKFVRSLGDNVTRMDRTEVQLNIPDGDLDTSTPQQLVANLRRLVLDEGLDSRGRDLLTDWLKRNTTGDQSIRAAVPAGWTVADKTGGGFKGETNDIAVIWPPGRAPIVMAVLTVPEDPTSTKGKPTIAAATRIVLRAFGA

SEQ ID NO: 32 - protein, 293 aa, Pseudomonas aeruginosa
  source 1..293: note = class A B-lactamase; note (original language) = B-lactamasa de clase A
MSLYRRLVLLSCLSWPLAGFSATALTNLVAEPFAKLEQDFGGSIGVYAMDTGSGATVSYRAEERFPLCSSFKGFLAAAVLARSQQQAGLLDTPIRYGKNALVPWSPISEKYLTTGMTVAELSAAAVQYSDNAAANLLLKELGGPAGLTAFMRSIGDTTFRLDRWELELNSAIPGDARDTSSPRAVTESLQKLTLGSALAAPQRQQFVDWLKGNTTGNHRIRAAVPADWAVGDKTGTCGVYGTANDYAVVWPTGRAPIVLAVYTRAPNKDDKHSEAVIAAAARLALEGLGVNGQ

SEQ ID NO: 33 - DNA, 984 bp, synthetic construct
  source 1..984: mol_type = other DNA; note = DNA coding for fragment of B-lactamase; note (original language) = ADN codificante para fragmento de B-lactamasa; organism (original language) = construccion sintetica
atgaaatacctgctgccgaccgctgctgctggtctgctgctcctcgctgcccagccggcgatggccatggatatcggaattaattcggatccggcgccggatgaactggcgagcctggaaaaagattttggcggccgcattggcgtgtatgcgctggataccggcagcggcgataccgtgggccatcgcgcggatgaacgctttctgatgtgcagcaccgtgaaaacctttattgtgagcgcgattctgcgccgccgcctgagcgaaccgggcctgctggatcagcgcattcagtatacccagagcgatgtgctggaatgggcgccgattaccagccagcatgtgagcaccggcatgaccgtgagcgaactgtgcgatgcgaccctgcgctatagcgataacaccggcgcgaacctgctgattacccagctgggcggcccgaaagaaaccgaaaaatttgtgcgcagcctgggcgataacgtgacccgcatggatcgcaccgaagtgcagctgaacattccggatggcgatctggataccagcaccccgcagcagctggtggcgaacctgcgccgcctggtgctggatgaaggcctggatagccgcggccgcgatctgctgaccgattggctgaaacgcaacaccaccggcgatcagagcattcgcgcggcggtgccggcgggctggaccgtggcggataaaaccggcggcggctttaaaggcgaaaccaacgatattgcggtgatttggccgccgggccgcgcgccgattgtgatggcggtgctgaccgtgccggaagatccgaccagcaccaaaggcaaaccgaccattgcggcggcgacccgcattgtgctgcgcgcgtttggcgcggaaaacctgtattttcagagcgattataaagatgatgatgataaagaggatccgaattcgagctccgtcgacaagcttgcggccgcactcgagcaccaccaccaccaccactga

SEQ ID NO: 34 - protein, 327 aa, synthetic construct
  source 1..327: note = Modified Class A B-lactamase M. abscessus; note (original language) = B-lactamasa de clase A de M. abscessus modificada; organism (original language) = construccion sintetica
MKYLLPTAAAGLLLLAAQPAMAMDIGINSDPAPDELASLEKDFGGRIGVYALDTGSGDTVGHRADERFLMCSTVKTFIVSAILRRRLSEPGLLDQRIQYTQSDVLEWAPITSQHVSTGMTVSELCDATLRYSDNTGANLLITQLGGPKETEKFVRSLGDNVTRMDRTEVQLNIPDGDLDTSTPQQLVANLRRLVLDEGLDSRGRDLLTDWLKRNTTGDQSIRAAVPAGWTVADKTGGGFKGETNDIAVIWPPGRAPIVMAVLTVPEDPTSTKGKPTIAAATRIVLRAFGAENLYFQSDYKDDDDKEDPNSSSVDKLAAALEHHHHHH

SEQ ID NO: 35 - protein, 307 aa, Mycobacterium tuberculosis
  source 1..307: note = Class A B-lactamase M.tuberculosis; note (original language) = B-lactamasa de clase A de M.tuberculosis
MRNRGFGRRELLVAMAMLVSVTGCARHASGARPASTTLPAGADLADRFAELERRYDARLGVYVPATGTTAAIEYRADERFAFCSTFKAPLVAAVLHQNPLTHLDKLITYTSDDIRSISPVAQQHVQTGMTIGQLCDAAIRYSDGTAANLLLADLGGPGGGTAAFTGYLRSLGDTVSRLDAEEPELNRDPPGDERDTTTPHAIALVLQQLVLGNALPPDKRALLTDWMARNTTGAKRIRAGFPADWKVIDKTGTGDYGRANDIAVVWSPTGVPYVVAVMSDRAGGGYDAEPREALLAEAATCVAGVLA

SEQ ID NO: 36 - protein, 306 aa, Listeria monocytogenes
  source 1..306: note = Class A B-lactamase Listeria monocytogenes; note (original language) = B-lactamasa de clase a Listeria monocytogenes
MRMRKILLGLTVIFAVAGLVACGAPDKNAAATKKEETKQETENAQVKAALEKLEKKYGATLGVYGMDMGGKQTISFNAEERFAYASTFKAIAGGILLKNLTDEQLNKRFTFSKEDLVDHSPITEKHVDSGMTMKELINASMTYSDNTAANLTLQQLGGPKGFEKELVKIGDKTMKPVRFEPELNDAVPGDIRDTTTPEAMAKTFAYLLTEGNLPADRLAYFKQTLIDNTTGATLIRAGVPAGYIVGDRTGAGSYGTRNAIAMIYPKDKDTKPLVWVIYSKKTGKDDEYNDQLIADAAKVLSDYYSL

SEQ ID NO: 37 - protein, 247 aa, Staphylococcus aureus
  source 1..247: note = Class A B-lactamase Staphylococcus aureus; note (original language) = B-lactamasa de clase A de Staphylococcus aureus
VKDAEDQLGARVGYIELDLNSGKILESFRPEERFPMMSTFKVLLCGAVLSRIDAGQEQLGRRIHYSQNDLVEYSPVTEKHLTDGMTVRELCSAAITMSDNTAANLLLTTIGGPKELTAFLHNMGDHVTRLDRWEPELNEAIPNDERDTTMPVAMATTLRKLLTGELLTLASRQQLIDWMEADKVAGPLLRSALPAGWFIADKSGAGERGSRGIIAALGPDGKPSRVVVIYTTGSQATMDERNRQIAE

SEQ ID NO: 38 - protein, 314 aa, Streptococcus pneumoniae
  source 1..314: note = Class A B-lactamase Streptococcus pneumoniae; note (original language) = B-lactamasa de clase A de Streptococcus pneumoniae
MYVLNKFFTYKKIVPVVLLSCVTLIGCSNSNTPSELPKQTKQIKQIKQENTRHDSFAKLEKEYNAKLGIYALDTGTNQTVAYHPNDRFAFASTSKSLAAGALLRQNSIEALDERITYTREDLSNYNPITEKHVDTGMTLKELADASVRYSDSTAHNLILKKLGGPSAFEKILRETGDTVTKSERFEPELNEVHPGETRDTSTPEAIAKTLQSFTLGSALPTEKRELLVDWMKRNTTGDKLIRAGVPKGWEVADKTGAGSYGTRNDIAIIWPPNKKPIVLAILSNHDKEDAEYDDKLIADATKVVLDTLKVTNKN

SEQ ID NO: 39 - protein, 281 aa, Clostridium difficile
  source 1..281: note = Class A B-lactamase Clostridium difficile; note (original language) = B-lactamasa de lcase A de Clostridium difficile
MKKLIFLIAIALVLSACNSNSSHAKELNDLEKKYNAHIGVYALDTKSGKEVKFNSDKRFAYASTSKAINSAILLEQVPYNKLNKKIHINKDDIVAYSPILEKYVGKDITLKELIEASMAYSDNTANNKIIKEIGGIKKVKQRLKELGDKVTNPVRYEIELNYYSPKSKKDTSTPAAFGKTLNKLIANGKLSKENKKFLLDLMLNNKSGDTLIKDGVSKDCKVADKSGQAITYASRNDVAFVYPKGQSEPIVLVIFTNKDNKSDKPNDKLISETAKSVMKEF

SEQ ID NO: 40 - protein, 311 aa, Bacillus anthracis
  source 1..311: note = Class A B-lactamase Bacillus anthracis; note (original language) = B-lactamasa de clase A de Bacillus anthracis
MIVLNKFFNMLPYKKIVPVLFLSCATLIGCSNSNTQSEPPKQAKQENTVNHSFAKLEKEFDAKLGIYALDTDTNQTVTYQSDERFAYASTHKALAVGVLLQKKSIEDLNQRILYTREDLVNYNPITEKYVDTGMTLKELADASLRYSDNTAQNLILKQLGGPSEFKKSLREIGDTVTNPERFEPELNEVHPGDTHDTSTPKALATSLQAFALGDILSTEKRNLLIDWMKRNTTGDKLIRAGVPGGWEVADKTGSGSYGTRNDIAIIWPPNKKPIVLAILSNQGKEDAKYDDKLIAEATKIVLHALKTPNKQ

SEQ ID NO: 41 - protein, 122 aa, synthetic construct
  source 1..122: note = control antibody D1.1; note (original language) = Anticuerpo control D1.1; organism (original language) = construccion sintetica
QVQLQESGGGLVQAGGSLRLSCAASGTISYSYSMGWYRQAPGKDREFVATIAAGGSTYYADSVKGRFTISRDNAKNTVYLQMNSLKPEDTAVYYCAVRYQPQPHPRVYHYYWGQGTQVTVSS

SEQ ID NO: 42 - protein, 7 aa, synthetic construct
  source 1..7: note = TEV protease recognition sequence; note (original language) = Secuenica de reconocimiento TEV proteasa; organism (original language) = construccion sintetica
ENLYFQS

SEQ ID NO: 43 - protein, 8 aa, synthetic construct
  source 1..8: note = tag; note (original language) = etiqueta; organism (original language) = construccion sintetica
DYKDDDDK

SEQ ID NO: 44 - protein, 25 aa, synthetic construct
  source 1..25: note = FR1 sequence; note (original language) = secuenica FR1; organism (original language) = construccion sintetica
QVQLQESGGGLVQAGGSLRLSCAAS

SEQ ID NO: 45 - protein, 12 aa, synthetic construct
  source 1..12: note = FR2 sequence; note (original language) = secuencia FR2; organism (original language) = construccion sintetica
MGWYRQAPGKER

SEQ ID NO: 46 - protein, 37 aa, synthetic construct
  source 1..37: note = FR3 sequence; note (original language) = secuencia FR3; organism (original language) = construccion sintetica
ADSVKGRFTISRDNAKNTVYLQMNSLKPEDTAVYYCA

SEQ ID NO: 47 - protein, 12 aa, synthetic construct
  source 1..12: note = FR4 sequence; note (original language) = seucuencia FR4; organism (original language) = construccion sintetica
YWGQGTQVTVSS